European Patent Application EP 4 567 115 A1, published June 11, 2025. Title: Method of producing ribosome in cell-free protein synthesis system. Applicant: Kyoto University. Application WO. The sequence listing filed with the application follows.

SEQUENCE LISTING (5 sequences)

SEQ ID NO: 1 - DNA, 60 bp, synthetic construct
  source 1..60: mol_type = other DNA
gaaattgtgagcggataacaatttcacacaggaaacagctgtgtaggctggagctgcttc

SEQ ID NO: 2 - DNA, 60 bp, synthetic construct
  source 1..60: mol_type = other DNA
ttacgcgaaatacgggcagacatggcctgcccggttattaattccggggatccgtcgacc

SEQ ID NO: 3 - DNA, 10278 bp, synthetic construct
  source 1..10278: mol_type = other DNA
gtcatcaccgaaacgcgcgaggcagctgcggtaaagctcatcagcgtggtcgtgaagcgattcacagatgtctgcctgttcatccgcgtccagctcgttgagtttctccagaagcgttaatgtctggcttctgataaagcgggccatgttaagggcggttttttcctgtttggtcactgatgcctccgtgtaagggggatttctgttcatgggggtaatgataccgatgaaacgagagaggatgctcacgatacgggttactgatgatgaacatgcccggttactggaacgttgtgagggtaaacaactggcggtatggatgcggcgggaccagagaaaaatcactcagggtcaatgccagcgcttcgttaatacagatgtaggtgttccacagggtagccagcagcatcctgcgatgcagatccggaacataatggtgcagggcgctgacttccgcgtttccagactttacgaaacacggaaaccgaagaccattcatgttgttgctcaggtcgcagacgttttgcagcagcagtcgcttcacgttcgctcgcgtatcggtgattcattctgctaaccagtaaggcaaccccgccagcctagccgggtcctcaacgacaggagcacgatcatgctagtcatgccccgcgcccaccggaaggagctgactgggttgaaggctctcaagggcatcggtcgagatcccggtgcctaatgagtgagctaacttacattaattgcgttgcgctcactgcccgctttccagtcgggaaacctgtcgtgccagctgcattaatgaatcggccaacgcgcggggagaggcggtttgcgtattgggcgccagggtggtttttcttttcaccagtgagacgggcaacagctgattgcccttcaccgcctggccctgagagagttgcagcaagcggtccacgctggtttgccccagcaggcgaaaatcctgtttgatggtggttaacggcgggatataacatgagctgtcttcggtatcgtcgtatcccactaccgagatgtccgcaccaacgcgcagcccggactcggtaatggcgcgcattgcgcccagcgccatctgatcgttggcaaccagcatcgcagtgggaacgatgccctcattcagcatttgcatggtttgttgaaaaccggacatggcactccagtcgccttcccgttccgctatcggctgaatttgattgcgagtgagatatttatgccagccagccagacgcagacgcgccgagacagaacttaatgggcccgctaacagcgcgatttgctggtgacccaatgcgaccagatgctccacgcccagtcgcgtaccgtcttcatgggagaaaataatactgttgatgggtgtctggtcagagacatcaagaaataacgccggaacattagtgcaggcagcttccacagcaatggcatcctggtcatccagcggatagttaatgatcagcccactgacgcgttgcgcgagaagattgtgcaccgccgctttacaggcttcgacgccgcttcgttctaccatcgacaccaccacgctggcacccagttgatcggcgcgagatttaatcgccgcgacaatttgcgacggcgcgtgcagggccagactggaggtggcaacgccaatcagcaacgactgtttgcccgccagttgttgtgccacgcggttgggaatgtaattcagctccgccatcgccgcttccactttttcccgcgttttcgcagaaacgtggctggcctggttcaccacgcgggaaacggtctgataagagacaccggcatactctgcgacatcgtataacgttactggtttcacattcaccaccctgaattgactctcttccgggcgctatcatgccataccgcgaaaggttttgcgccattcgatggtgtccgggatctcgacgctctcccttatgcgactcctgcattaggaagcagcccagtagtaggttgaggccgttgagcaccgccgccgcaaggaatggtgcatgcaaggagatggcgcccaacagtcccccggccacggggcctgccaccatacccacgccgaaacaagcgctcatgagcccgaagtggcgagcccgatcttccccatcggtgatgtcggcgatataggcgccagcaaccgcacctgtggcgccggtgatgccggccacgatgcgtccggcgtagaggatcgagatcgatctcgatcccgcgaaattaatacgactcactataggggaattgtgagcggataacaattcccctctagaaataattttgtttaactttaagaaggagatatacatagcgccgctgagaaaaagcgaagcggcactgctctttaacaatttatcagacaatctgtgtgggcactcgaagatacggattcttaacgtcgcaagacgaaaaatgaataccaagtctcaagagtgaacacgtaattcattacgaagtttaattctttgagcgtcaaacttttaaattgaagagtttgatcatggctcagattgaacgctggcggcaggcctaacacatgcaagtcgaacggtaacaggaagaagcttgcttctttgctgacgagtggcggacgggtgagtaatgtctgggaaactgcctgatggagggggataactactggaaacggtagctaataccgcataacgtcgcaagaccaaagagggggaccttcgggcctcttgccatcggatgtgcccagatgggattagctagtaggtggggtaacggctcacctaggcgacgatccctagctggtctgagaggatgaccagccacactggaactgagacacggtccagactcctacgggaggcagcagtggggaatattgcacaatgggcgcaagcctgatgcagccatgccgcgtgtatgaagaaggccttcgggttgtaaagtactttcagcggggaggaagggagtaaagttaatacctttgctcattgacgttacccgcagaagaagcaccggctaactccgtgccagcagccgcggtaatacggagggtgcaagcgttaatcggaattactgggcgtaaagcgcacgcaggcggtttgttaagtcagatgtgaaatccccgggctcaacctgggaactgcatctgatactggcaagcttgagtctcgtagaggggggtagaattccaggtgtagcggtgaaatgcgtagagatctggaggaataccggtggcgaaggcggccccctggacgaagactgacgctcaggtgcgaaagcgtggggagcaaacaggattagataccctggtagtccacgccgtaaacgatgtcgacttggaggttgtgcccttgaggcgtggcttccggagctaacgcgttaagtcgaccgcctggggagtacggccgcaaggttaaaactcaaatgaattgacgggggcccgcacaagcggtggagcatgtggtttaattcgatgcaacgcgaagaaccttacctggtcttgacatccacggaagttttcagagatgagaatgtgccttcctcgagcccgaccagaatcatgcaagtgcgtaagatagtcgcgggccgggctagcgggaaccgtgagacaggtgctgcatggctgtcgtcagctcgtgttgtgaaatgttgggttaagtcccgcaacgagcgcaacccttatcctttgttgccagcggtccggccgggaactcaaaggagactgccagtgataaactggaggaaggtggggatgatgtcaagtcatcatggcccttacgaccagggctacacacgtgctacaatggcgcatacaaagagaagcgacctcgcgagagcaagcggacctcataaagtgcgtcgtagtccggattggagtctgcaactcgactccatgaagtcggaatcgctagtaatcgtggatcagaatgccacggtgaatacgttcccgggccttgtacacaccgcccgtcacaccatgggagtgggttgcaaaagaagtaggtagcttaaccttcgggagggcgcttaccactttgtgattcatgactggggtgaagtcgtaacaaggtaaccgtaggggaacctgcggttggatcacgagactaccttaaagaagcgtactttgtagtgctcacacagattgtctgatagaaagtgaaaagcaaggcgtttacgcgttgggagtgaggctgaagagaataaggccgttcgctttctattaatgaaagctcaccctacacgaaaatatcacgcaacgcgtgataagcaattttcgtgtccccttcgtctagaggcccaggacaccgccctttcacggcggtaacaggggttcgaatcccctaggggacgccacttgctggtttgtgagtgaaagtcgccgaccttaatatctcaaaactcatcttcgggtgatgtttgagatatttgctctttaaaaatctggatcaagctgaaaattgaaacactgaacaacgagagttgttcgtgagtctctcaaattttcgcaacacgatgatgaatcgaaagaaacatcttcgggttgtgaggttaagcgactaagcgtacacggtggatgccctggcagtcagaggcgatgaaggacgtgctaatctgcgataagcgtcggtaaggtgatatgaaccgttataaccggcgatttccgaatggggaaacccagtgtgtttcgacacactatcattaactgaatccataggttaatgaggcgaaccgggggaactgaaacatctaagtaccccgaggaaaagaaatcaaccgagattcccccagtagcggcgagcgaacggggagcagcccagagcctgaatcagtgtgtgtgttagtggaagcgtctggaaaggcgcgcgatacagggtgacagccccgtacacaaaaatgcacatgctgtgagctcgatgagtagggcgggacacgtggtatcctgtctgaatatggggggaccatcctccaaggctaaatactcctgactgaccgatagtgaaccagtaccgtgagggaaaggcgaaaagaaccccggcgaggggagtgaaaaagaacctgaaaccgtgtacgtacaagcagtgggagcacgcttaggcgtgtgactgcgtaccttttgtataatgggtcagcgacttatattctgtagcaaggttaaccgaataggggagccgaagggaaaccgagtcttaactgggcgttaagttgcagggtatagacccgaaacccggtgatctagccatgggcaggttgaaggttgggtaacactaactggaggaccgaaccgactaatgttgaaaaattagcggatgacttgtggctgggggtgaaaggccaatcaaaccgggagatagctggttctccccgaaagctatttaggtagcgcctcgtgaattcatctccgggggtagagcactgtttcggcaagggggtcatcccgacttaccaacccgatgcaaactgcgaataccggagaatgttatcacgggagacacacggcgggtgctaacgtccgtcgtgaagagggaaacaacccagaccgccagctaaggtcccaaagtcatggttaagtgggaaacgatgtgggaaggcccagacagccaggatgttggcttagaagcagccatcatttaaagaaagcgtaatagctcactggtcgagtcggcctgcgcggaagatgtaacggggctaaaccatgcaccgaagctgcggcagcgacgcttatgcgttgttgggtaggggagcgttctgtaagcctgcgaaggtgtgctgtgaggcatgctggaggtatcagaagtgcgaatgctgacataagtaacgataaagcgggtgaaaagcccgctcgccggaagaccaagggttcctgtccaacgttaatcggggcagggtgagtcgacccctaaggcgaggccgaaaggcgtagtcgatgggaaacaggttaatattcctgtacttggtgttactgcgaaggggggacggagaaggctatgttggccgggcgacggttgtcccggtttaagcgtgtaggctggttttccaggcaaatccggaaaatcaaggctgaggcgtgatgacgaggcactacggtgctgaagcaacaaatgccctgcttccaggaaaagcctctaagcatcaggtaacatcaaatcgtaccccaaaccgacacaggtggtcaggtagagaataccaaggcgcttgagagaactcgggtgaaggaactaggcaaaatggtgccgtaacttcgggagaaggcacgctgatatgtaggtgaggtccctcgcggatggagctgaaatcagtcgaagataccagctggctgcaactgtttattaaaaacacagcactgtgcaaacacgaaagtggacgtatacggtgtgacgcctgcccggtgccggaaggttaattgatggggttagcgcaagcgaagctcttgatcgaagccccggtaaacggcggccgtaactataacggtcctaaggtagcgaaattccttgtcgggtaagttccgacctgcacgaatggcgtaatgatggccaggctgtctccacccgagactcagtgaaattgaactcgctgtgaagatgcagtgtacccgcggcaagacggtaagaccccgtgaacctttactatagcttgacactgaacattgagccttgatgtgtaggataggtgggaggctttgaagtgtggacgccagtctgcatggagccgaccttgaaataccaccctttaatgtttgatgttctaacgttgacccgtaatccgggttgcggacagtgtctggtgggtagtttgactggggcggtctcctcctaaagagtaacggaggagcacgaaggttggctaatcctggtcggacatcaggaggttagtgcaatggcataagccagcttgactgcgagcgtgacggcgcgagcaggtgcgaaagcaggtcatagtgatccggtggttctgaatggaagggccatcgctcaacggataaaaggtactccggggataacaggctgataccgcccaagagttcatatcgacggcggtgtttggcacctcgatgtcggctcatcacatcctggggctgaagtaggtcccaagggtatggctgttcgccatttaaagtggtacgcgagctgggtttagaacgtcgtgagacagttcggtccctatctgccgtgggcgctggagaactgaggggggctgctcctagtacgagaggaccggagtggacgcatcactggtgttcgggttgtcatgccaatggcactgcccggtagctaaatgcggaagagataagtgctgaaagcatctaagcacgaaacttgccccgagatgagttctccctgaccctttaagggtcctgaaggaacgttgaagacgacgacgttgataggccgggtgtgtaagcgcagcgatgcgttgagctaaccggtactaatgaaccgtgaggcttaaccttacaacgccgaagctgttttggcggatgagagaagattttcagcctgatacagattaaatcagaacgcagaagcggtctgataaaacagaatttgcctggcggcagtagcgcggtggtcccacctgaccccatgccgaactcagaagtgaaacgccgtagcgccgatggtagtgtggggtctccccatgcgagagtagggaactgccaggcatcaaataaagctgagttggctgctgccaccgctgagcaataactagcataaccccttggggcctctaaacgggtcttgaggggttttttgctgaaaggaggaactatatccggattggcgaatgggacgcgccctgtagcggcgcattaagcgcggcgggtgtggtggttacgcgcagcgtgaccgctacacttgccagcgccctagcgcccgctcctttcgctttcttcccttcctttctcgccacgttcgccggctttccccgtcaagctctaaatcgggggctccctttagggttccgatttagtgctttacggcacctcgaccccaaaaaacttgattagggtgatggttcacgtagtgggccatcgccctgatagacggtttttcgccctttgacgttggagtccacgttctttaatagtggactcttgttccaaactggaacaacactcaaccctatctcggtctattcttttgatttataagggattttgccgatttcggcctattggttaaaaaatgagctgatttaacaaaaatttaacgcgaattttaacaaaatattaacgtttacaatttcaggtggcacttttcggggaaatgtgcgcggaacccctatttgtttatttttctaaatacattcaaatatgtatccgctcatgaattaattcttagaaaaactcatcgagcatcaaatgaaactgcaatttattcatatcaggattatcaataccatatttttgaaaaagccgtttctgtaatgaaggagaaaactcaccgaggcagttccataggatggcaagatcctggtatcggtctgcgattccgactcgtccaacatcaatacaacctattaatttcccctcgtcaaaaataaggttatcaagtgagaaatcaccatgagtgacgactgaatccggtgagaatggcaaaagtttatgcatttctttccagacttgttcaacaggccagccattacgctcgtcatcaaaatcactcgcatcaaccaaaccgttattcattcgtgattgcgcctgagcgagacgaaatacgcgatcgctgttaaaaggacaattacaaacaggaatcgaatgcaaccggcgcaggaacactgccagcgcatcaacaatattttcacctgaatcaggatattcttctaatacctggaatgctgttttcccggggatcgcagtggtgagtaaccatgcatcatcaggagtacggataaaatgcttgatggtcggaagaggcataaattccgtcagccagtttagtctgaccatctcatctgtaacatcattggcaacgctacctttgccatgtttcagaaacaactctggcgcatcgggcttcccatacaatcgatagattgtcgcacctgattgcccgacattatcgcgagcccatttatacccatataaatcagcatccatgttggaatttaatcgcggcctagagcaagacgtttcccgttgaatatggctcataacaccccttgtattactgtttatgtaagcagacagttttattgttcatgaccaaaatcccttaacgtgagttttcgttccactgagcgtcagaccccgtagaaaagatcaaaggatcttcttgagatcctttttttctgcgcgtaatctgctgcttgcaaacaaaaaaaccaccgctaccagcggtggtttgtttgccggatcaagagctaccaactctttttccgaaggtaactggcttcagcagagcgcagataccaaatactgtccttctagtgtagccgtagttaggccaccacttcaagaactctgtagcaccgcctacatacctcgctctgctaatcctgttaccagtggctgctgccagtggcgataagtcgtgtcttaccgggttggactcaagacgatagttaccggataaggcgcagcggtcgggctgaacggggggttcgtgcacacagcccagcttggagcgaacgacctacaccgaactgagatacctacagcgtgagctatgagaaagcgccacgcttcccgaagggagaaaggcggacaggtatccggtaagcggcagggtcggaacaggagagcgcacgagggagcttccagggggaaacgcctggtatctttatagtcctgtcgggtttcgccacctctgacttgagcgtcgatttttgtgatgctcgtcaggggggcggagcctatggaaaaacgccagcaacgcggcctttttacggttcctggccttttgctggccttttgctcacatgttctttcctgcgttatcccctgattctgtggataaccgtattaccgcctttgagtgagctgataccgctcgccgcagccgaacgaccgagcgcagcgagtcagtgagcgaggaagcggaagagcgcctgatgcggtattttctccttacgcatctgtgcggtatttcacaccgcatatatggtgcactctcagtacaatctgctctgatgccgcatagttaagccagtatacactccgctatcgctacgtgactgggtcatggctgcgccccgacacccgccaacacccgctgacgcgccctgacgggcttgtctgctcccggcatccgcttacagacaagctgtgaccgtctccgggagctgcatgtgtcagaggttttcacc

SEQ ID NO: 4 - DNA, 10294 bp, synthetic construct
  source 1..10294: mol_type = other DNA
gtcatcaccgaaacgcgcgaggcagctgcggtaaagctcatcagcgtggtcgtgaagcgattcacagatgtctgcctgttcatccgcgtccagctcgttgagtttctccagaagcgttaatgtctggcttctgataaagcgggccatgttaagggcggttttttcctgtttggtcactgatgcctccgtgtaagggggatttctgttcatgggggtaatgataccgatgaaacgagagaggatgctcacgatacgggttactgatgatgaacatgcccggttactggaacgttgtgagggtaaacaactggcggtatggatgcggcgggaccagagaaaaatcactcagggtcaatgccagcgcttcgttaatacagatgtaggtgttccacagggtagccagcagcatcctgcgatgcagatccggaacataatggtgcagggcgctgacttccgcgtttccagactttacgaaacacggaaaccgaagaccattcatgttgttgctcaggtcgcagacgttttgcagcagcagtcgcttcacgttcgctcgcgtatcggtgattcattctgctaaccagtaaggcaaccccgccagcctagccgggtcctcaacgacaggagcacgatcatgctagtcatgccccgcgcccaccggaaggagctgactgggttgaaggctctcaagggcatcggtcgagatcccggtgcctaatgagtgagctaacttacattaattgcgttgcgctcactgcccgctttccagtcgggaaacctgtcgtgccagctgcattaatgaatcggccaacgcgcggggagaggcggtttgcgtattgggcgccagggtggtttttcttttcaccagtgagacgggcaacagctgattgcccttcaccgcctggccctgagagagttgcagcaagcggtccacgctggtttgccccagcaggcgaaaatcctgtttgatggtggttaacggcgggatataacatgagctgtcttcggtatcgtcgtatcccactaccgagatgtccgcaccaacgcgcagcccggactcggtaatggcgcgcattgcgcccagcgccatctgatcgttggcaaccagcatcgcagtgggaacgatgccctcattcagcatttgcatggtttgttgaaaaccggacatggcactccagtcgccttcccgttccgctatcggctgaatttgattgcgagtgagatatttatgccagccagccagacgcagacgcgccgagacagaacttaatgggcccgctaacagcgcgatttgctggtgacccaatgcgaccagatgctccacgcccagtcgcgtaccgtcttcatgggagaaaataatactgttgatgggtgtctggtcagagacatcaagaaataacgccggaacattagtgcaggcagcttccacagcaatggcatcctggtcatccagcggatagttaatgatcagcccactgacgcgttgcgcgagaagattgtgcaccgccgctttacaggcttcgacgccgcttcgttctaccatcgacaccaccacgctggcacccagttgatcggcgcgagatttaatcgccgcgacaatttgcgacggcgcgtgcagggccagactggaggtggcaacgccaatcagcaacgactgtttgcccgccagttgttgtgccacgcggttgggaatgtaattcagctccgccatcgccgcttccactttttcccgcgttttcgcagaaacgtggctggcctggttcaccacgcgggaaacggtctgataagagacaccggcatactctgcgacatcgtataacgttactggtttcacattcaccaccctgaattgactctcttccgggcgctatcatgccataccgcgaaaggttttgcgccattcgatggtgtccgggatctcgacgctctcccttatgcgactcctgcattaggaagcagcccagtagtaggttgaggccgttgagcaccgccgccgcaaggaatggtgcatgcaaggagatggcgcccaacagtcccccggccacggggcctgccaccatacccacgccgaaacaagcgctcatgagcccgaagtggcgagcccgatcttccccatcggtgatgtcggcgatataggcgccagcaaccgcacctgtggcgccggtgatgccggccacgatgcgtccggcgtagaggatcgagatcgatctcgatcccgcgaaattaatacgactcactataggggaattgtgagcggataacaattcccctctagaaataattttgtttaactttaagaaggagatatacatagcgccgctgagaaaaagcgaagcggcactgctctttaacaatttatcagacaatctgtgtgggcactcgaagatacggattcttaacgtcgcaagacgaaaaatgaataccaagtctcaagagtgaacacgtaattcattacgaagtttaattctttgagcgtcaaacttttaaattgaagagtttgatcatggctcagattgaacgctggcggcaggcctaacacatgcaagtcgaacggtaacaggaagaagcttgcttctttgctgacgagtggcggacgggtgagtaatgtctgggaaactgcctgatggagggggataactactggaaacggtagctaataccgcataacgtcgcaagaccaaagagggggaccttcgggcctcttgccatcggatgtgcccagatgggattagctagtaggtggggtaacggctcacctaggcgacgatccctagctggtctgagaggatgaccagccacactggaactgagacacggtccagactcctacgggaggcagcagtggggaatattgcacaatgggcgcaagcctgatgcagccatgccgcgtgtatgaagaaggccttcgggttgtaaagtactttcagcggggaggaagggagtaaagttaatacctttgctcattgacgttacccgcagaagaagcaccggctaactccgtgccagcagccgcggtaatacggagggtgcaagcgttaatcggaattactgggcgtaaagcgcacgcaggcggtttgttaagtcagatgtgaaatccccgggctcaacctgggaactgcatctgatactggcaagcttgagtctcgtagaggggggtagaattccaggtgtagcggtgaaatgcgtagagatctggaggaataccggtggcgaaggcggccccctggacgaagactgacgctcaggtgcgaaagcgtggggagcaaacaggattagataccctggtagtccacgccgtaaacgatgtcgacttggaggttgtgcccttgaggcgtggcttccggagctaacgcgttaagtcgaccgcctggggagtacggccgcaaggttaaaactcaaatgaattgacgggggcccgcacaagcggtggagcatgtggtttaattcgatgcaacgcgaagaaccttacctggtcttgacatccacggaagttttcagagatgagaatgtgccttcgggaaccgtgagacaggtgctgcatggctgtcgtcagctcgtgttgtgaaatgttgggttaagtcccgcaacgagcgcaacccttatcctttgttgccagcggtccggccgggaactcaaaggagactgccagtgataaactggaggaaggtggggatgatgtcaagtcatcatggcccttacgaccagggctacacacgtgctacaatggcgcatacaaagagaagcgacctcgcgagagcaagcggacctcataaagtgcgtcgtagtccggattggagtctgcaactcgactccatgaagtcggaatcgctagtaatcgtggatcagaatgccacggtgaatacgttcccgggccttgtacacaccgcccgtcacaccatgggagtgggttgcaaaagaagtaggtagcttaaccttcgggagggcgcttaccactttgtgattcatgactggggtgaagtcgtaacaaggtaaccgtaggggaacctgcggttggatcacgagactaccttaaagaagcgtactttgtagtgctcacacagattgtctgatagaaagtgaaaagcaaggcgtttacgcgttgggagtgaggctgaagagaataaggccgttcgctttctattaatgaaagctcaccctacacgaaaatatcacgcaacgcgtgataagcaattttcgtgtccccttcgtctagaggcccaggacaccgccctttcacggcggtaacaggggttcgaatcccctaggggacgccacttgctggtttgtgagtgaaagtcgccgaccttaatatctcaaaactcatcttcgggtgatgtttgagatatttgctctttaaaaatctggatcaagctgaaaattgaaacactgaacaacgagagttgttcgtgagtctctcaaattttcgcaacacgatgatgaatcgaaagaaacatcttcgggttgtgaggttaagcgactaagcgtacacggtggatgccctggcagtcagaggcgatgaaggacgtgctaatctgcgataagcgtcggtaaggtgatatgaaccgttataaccggcgatttccgaatggggaaacccagtgtgtttcgacacactatcattaactgaatccataggttaatgaggcgaaccgggggaactgaaacatctaagtaccccgaggaaaagaaatcaaccgagattcccccagtagcggcgagcgaacggggagcagcccagagcctgaatcagtgtgtgtgttagtggaagcgtctggaaaggcgcgcgatacagggtgacagccccgtacacaaaaatgcacatgctgtgagctcgatgagtagggcgggacacgtggtatcctgtctgaatatggggggaccatcctccaaggctaaatactcctgactgaccgatagtgaaccagtaccgtgagggaaaggcgaaaagaaccccggcgaggggagtgaaaaagaacctgaaaccgtgtacgtacaagcagtgggagcacgcttgggtaccggctgggccgaccagaatcatgcaagtgcgtaagatagtcgcgggccggcccggccgggtactcaggcgtgtgactgcgtaccttttgtataatgggtcagcgacttatattctgtagcaaggttaaccgaataggggagccgaagggaaaccgagtcttaactgggcgttaagttgcagggtatagacccgaaacccggtgatctagccatgggcaggttgaaggttgggtaacactaactggaggaccgaaccgactaatgttgaaaaattagcggatgacttgtggctgggggtgaaaggccaatcaaaccgggagatagctggttctccccgaaagctatttaggtagcgcctcgtgaattcatctccgggggtagagcactgtttcggcaagggggtcatcccgacttaccaacccgatgcaaactgcgaataccggagaatgttatcacgggagacacacggcgggtgctaacgtccgtcgtgaagagggaaacaacccagaccgccagctaaggtcccaaagtcatggttaagtgggaaacgatgtgggaaggcccagacagccaggatgttggcttagaagcagccatcatttaaagaaagcgtaatagctcactggtcgagtcggcctgcgcggaagatgtaacggggctaaaccatgcaccgaagctgcggcagcgacgcttatgcgttgttgggtaggggagcgttctgtaagcctgcgaaggtgtgctgtgaggcatgctggaggtatcagaagtgcgaatgctgacataagtaacgataaagcgggtgaaaagcccgctcgccggaagaccaagggttcctgtccaacgttaatcggggcagggtgagtcgacccctaaggcgaggccgaaaggcgtagtcgatgggaaacaggttaatattcctgtacttggtgttactgcgaaggggggacggagaaggctatgttggccgggcgacggttgtcccggtttaagcgtgtaggctggttttccaggcaaatccggaaaatcaaggctgaggcgtgatgacgaggcactacggtgctgaagcaacaaatgccctgcttccaggaaaagcctctaagcatcaggtaacatcaaatcgtaccccaaaccgacacaggtggtcaggtagagaataccaaggcgcttgagagaactcgggtgaaggaactaggcaaaatggtgccgtaacttcgggagaaggcacgctgatatgtaggtgaggtccctcgcggatggagctgaaatcagtcgaagataccagctggctgcaactgtttattaaaaacacagcactgtgcaaacacgaaagtggacgtatacggtgtgacgcctgcccggtgccggaaggttaattgatggggttagcgcaagcgaagctcttgatcgaagccccggtaaacggcggccgtaactataacggtcctaaggtagcgaaattccttgtcgggtaagttccgacctgcacgaatggcgtaatgatggccaggctgtctccacccgagactcagtgaaattgaactcgctgtgaagatgcagtgtacccgcggcaagacggtaagaccccgtgaacctttactatagcttgacactgaacattgagccttgatgtgtaggataggtgggaggctttgaagtgtggacgccagtctgcatggagccgaccttgaaataccaccctttaatgtttgatgttctaacgttgacccgtaatccgggttgcggacagtgtctggtgggtagtttgactggggcggtctcctcctaaagagtaacggaggagcacgaaggttggctaatcctggtcggacatcaggaggttagtgcaatggcataagccagcttgactgcgagcgtgacggcgcgagcaggtgcgaaagcaggtcatagtgatccggtggttctgaatggaagggccatcgctcaacggataaaaggtactccggggataacaggctgataccgcccaagagttcatatcgacggcggtgtttggcacctcgatgtcggctcatcacatcctggggctgaagtaggtcccaagggtatggctgttcgccatttaaagtggtacgcgagctgggtttagaacgtcgtgagacagttcggtccctatctgccgtgggcgctggagaactgaggggggctgctcctagtacgagaggaccggagtggacgcatcactggtgttcgggttgtcatgccaatggcactgcccggtagctaaatgcggaagagataagtgctgaaagcatctaagcacgaaacttgccccgagatgagttctccctgaccctttaagggtcctgaaggaacgttgaagacgacgacgttgataggccgggtgtgtaagcgcagcgatgcgttgagctaaccggtactaatgaaccgtgaggcttaaccttacaacgccgaagctgttttggcggatgagagaagattttcagcctgatacagattaaatcagaacgcagaagcggtctgataaaacagaatttgcctggcggcagtagcgcggtggtcccacctgaccccatgccgaactcagaagtgaaacgccgtagcgccgatggtagtgtggggtctccccatgcgagagtagggaactgccaggcatcaaataaagctgagttggctgctgccaccgctgagcaataactagcataaccccttggggcctctaaacgggtcttgaggggttttttgctgaaaggaggaactatatccggattggcgaatgggacgcgccctgtagcggcgcattaagcgcggcgggtgtggtggttacgcgcagcgtgaccgctacacttgccagcgccctagcgcccgctcctttcgctttcttcccttcctttctcgccacgttcgccggctttccccgtcaagctctaaatcgggggctccctttagggttccgatttagtgctttacggcacctcgaccccaaaaaacttgattagggtgatggttcacgtagtgggccatcgccctgatagacggtttttcgccctttgacgttggagtccacgttctttaatagtggactcttgttccaaactggaacaacactcaaccctatctcggtctattcttttgatttataagggattttgccgatttcggcctattggttaaaaaatgagctgatttaacaaaaatttaacgcgaattttaacaaaatattaacgtttacaatttcaggtggcacttttcggggaaatgtgcgcggaacccctatttgtttatttttctaaatacattcaaatatgtatccgctcatgaattaattcttagaaaaactcatcgagcatcaaatgaaactgcaatttattcatatcaggattatcaataccatatttttgaaaaagccgtttctgtaatgaaggagaaaactcaccgaggcagttccataggatggcaagatcctggtatcggtctgcgattccgactcgtccaacatcaatacaacctattaatttcccctcgtcaaaaataaggttatcaagtgagaaatcaccatgagtgacgactgaatccggtgagaatggcaaaagtttatgcatttctttccagacttgttcaacaggccagccattacgctcgtcatcaaaatcactcgcatcaaccaaaccgttattcattcgtgattgcgcctgagcgagacgaaatacgcgatcgctgttaaaaggacaattacaaacaggaatcgaatgcaaccggcgcaggaacactgccagcgcatcaacaatattttcacctgaatcaggatattcttctaatacctggaatgctgttttcccggggatcgcagtggtgagtaaccatgcatcatcaggagtacggataaaatgcttgatggtcggaagaggcataaattccgtcagccagtttagtctgaccatctcatctgtaacatcattggcaacgctacctttgccatgtttcagaaacaactctggcgcatcgggcttcccatacaatcgatagattgtcgcacctgattgcccgacattatcgcgagcccatttatacccatataaatcagcatccatgttggaatttaatcgcggcctagagcaagacgtttcccgttgaatatggctcataacaccccttgtattactgtttatgtaagcagacagttttattgttcatgaccaaaatcccttaacgtgagttttcgttccactgagcgtcagaccccgtagaaaagatcaaaggatcttcttgagatcctttttttctgcgcgtaatctgctgcttgcaaacaaaaaaaccaccgctaccagcggtggtttgtttgccggatcaagagctaccaactctttttccgaaggtaactggcttcagcagagcgcagataccaaatactgtccttctagtgtagccgtagttaggccaccacttcaagaactctgtagcaccgcctacatacctcgctctgctaatcctgttaccagtggctgctgccagtggcgataagtcgtgtcttaccgggttggactcaagacgatagttaccggataaggcgcagcggtcgggctgaacggggggttcgtgcacacagcccagcttggagcgaacgacctacaccgaactgagatacctacagcgtgagctatgagaaagcgccacgcttcccgaagggagaaaggcggacaggtatccggtaagcggcagggtcggaacaggagagcgcacgagggagcttccagggggaaacgcctggtatctttatagtcctgtcgggtttcgccacctctgacttgagcgtcgatttttgtgatgctcgtcaggggggcggagcctatggaaaaacgccagcaacgcggcctttttacggttcctggccttttgctggccttttgctcacatgttctttcctgcgttatcccctgattctgtggataaccgtattaccgcctttgagtgagctgataccgctcgccgcagccgaacgaccgagcgcagcgagtcagtgagcgaggaagcggaagagcgcctgatgcggtattttctccttacgcatctgtgcggtatttcacaccgcatatatggtgcactctcagtacaatctgctctgatgccgcatagttaagccagtatacactccgctatcgctacgtgactgggtcatggctgcgccccgacacccgccaacacccgctgacgcgccctgacgggcttgtctgctcccggcatccgcttacagacaagctgtgaccgtctccgggagctgcatgtgtcagaggttttcacc

SEQ ID NO: 5 - DNA, 10349 bp, synthetic construct
  source 1..10349: mol_type = other DNA
gtcatcaccgaaacgcgcgaggcagctgcggtaaagctcatcagcgtggtcgtgaagcgattcacagatgtctgcctgttcatccgcgtccagctcgttgagtttctccagaagcgttaatgtctggcttctgataaagcgggccatgttaagggcggttttttcctgtttggtcactgatgcctccgtgtaagggggatttctgttcatgggggtaatgataccgatgaaacgagagaggatgctcacgatacgggttactgatgatgaacatgcccggttactggaacgttgtgagggtaaacaactggcggtatggatgcggcgggaccagagaaaaatcactcagggtcaatgccagcgcttcgttaatacagatgtaggtgttccacagggtagccagcagcatcctgcgatgcagatccggaacataatggtgcagggcgctgacttccgcgtttccagactttacgaaacacggaaaccgaagaccattcatgttgttgctcaggtcgcagacgttttgcagcagcagtcgcttcacgttcgctcgcgtatcggtgattcattctgctaaccagtaaggcaaccccgccagcctagccgggtcctcaacgacaggagcacgatcatgctagtcatgccccgcgcccaccggaaggagctgactgggttgaaggctctcaagggcatcggtcgagatcccggtgcctaatgagtgagctaacttacattaattgcgttgcgctcactgcccgctttccagtcgggaaacctgtcgtgccagctgcattaatgaatcggccaacgcgcggggagaggcggtttgcgtattgggcgccagggtggtttttcttttcaccagtgagacgggcaacagctgattgcccttcaccgcctggccctgagagagttgcagcaagcggtccacgctggtttgccccagcaggcgaaaatcctgtttgatggtggttaacggcgggatataacatgagctgtcttcggtatcgtcgtatcccactaccgagatgtccgcaccaacgcgcagcccggactcggtaatggcgcgcattgcgcccagcgccatctgatcgttggcaaccagcatcgcagtgggaacgatgccctcattcagcatttgcatggtttgttgaaaaccggacatggcactccagtcgccttcccgttccgctatcggctgaatttgattgcgagtgagatatttatgccagccagccagacgcagacgcgccgagacagaacttaatgggcccgctaacagcgcgatttgctggtgacccaatgcgaccagatgctccacgcccagtcgcgtaccgtcttcatgggagaaaataatactgttgatgggtgtctggtcagagacatcaagaaataacgccggaacattagtgcaggcagcttccacagcaatggcatcctggtcatccagcggatagttaatgatcagcccactgacgcgttgcgcgagaagattgtgcaccgccgctttacaggcttcgacgccgcttcgttctaccatcgacaccaccacgctggcacccagttgatcggcgcgagatttaatcgccgcgacaatttgcgacggcgcgtgcagggccagactggaggtggcaacgccaatcagcaacgactgtttgcccgccagttgttgtgccacgcggttgggaatgtaattcagctccgccatcgccgcttccactttttcccgcgttttcgcagaaacgtggctggcctggttcaccacgcgggaaacggtctgataagagacaccggcatactctgcgacatcgtataacgttactggtttcacattcaccaccctgaattgactctcttccgggcgctatcatgccataccgcgaaaggttttgcgccattcgatggtgtccgggatctcgacgctctcccttatgcgactcctgcattaggaagcagcccagtagtaggttgaggccgttgagcaccgccgccgcaaggaatggtgcatgcaaggagatggcgcccaacagtcccccggccacggggcctgccaccatacccacgccgaaacaagcgctcatgagcccgaagtggcgagcccgatcttccccatcggtgatgtcggcgatataggcgccagcaaccgcacctgtggcgccggtgatgccggccacgatgcgtccggcgtagaggatcgagatcgatctcgatcccgcgaaattaatacgactcactataggggaattgtgagcggataacaattcccctctagaaataattttgtttaactttaagaaggagatatacatagcgccgctgagaaaaagcgaagcggcactgctctttaacaatttatcagacaatctgtgtgggcactcgaagatacggattcttaacgtcgcaagacgaaaaatgaataccaagtctcaagagtgaacacgtaattcattacgaagtttaattctttgagcgtcaaacttttaaattgaagagtttgatcatggctcagattgaacgctggcggcaggcctaacacatgcaagtcgaacggtaacaggaagaagcttgcttctttgctgacgagtggcggacgggtgagtaatgtctgggaaactgcctgatggagggggataactactggaaacggtagctaataccgcataacgtcgcaagaccaaagagggggaccttcgggcctcttgccatcggatgtgcccagatgggattagctagtaggtggggtaacggctcacctaggcgacgatccctagctggtctgagaggatgaccagccacactggaactgagacacggtccagactcctacgggaggcagcagtggggaatattgcacaatgggcgcaagcctgatgcagccatgccgcgtgtatgaagaaggccttcgggttgtaaagtactttcagcggggaggaagggagtaaagttaatacctttgctcattgacgttacccgcagaagaagcaccggctaactccgtgccagcagccgcggtaatacggagggtgcaagcgttaatcggaattactgggcgtaaagcgcacgcaggcggtttgttaagtcagatgtgaaatccccgggctcaacctgggaactgcatctgatactggcaagcttgagtctcgtagaggggggtagaattccaggtgtagcggtgaaatgcgtagagatctggaggaataccggtggcgaaggcggccccctggacgaagactgacgctcaggtgcgaaagcgtggggagcaaacaggattagataccctggtagtccacgccgtaaacgatgtcgacttggaggttgtgcccttgaggcgtggcttccggagctaacgcgttaagtcgaccgcctggggagtacggccgcaaggttaaaactcaaatgaattgacgggggcccgcacaagcggtggagcatgtggtttaattcgatgcaacgcgaagaaccttacctggtcttgacatccacggaagttttcagagatgagaatgtgccttcctcgagcccgaccagaatcatgcaagtgcgtaagatagtcgcgggccgggctagcgggaaccgtgagacaggtgctgcatggctgtcgtcagctcgtgttgtgaaatgttgggttaagtcccgcaacgagcgcaacccttatcctttgttgccagcggtccggccgggaactcaaaggagactgccagtgataaactggaggaaggtggggatgatgtcaagtcatcatggcccttacgaccagggctacacacgtgctacaatggcgcatacaaagagaagcgacctcgcgagagcaagcggacctcataaagtgcgtcgtagtccggattggagtctgcaactcgactccatgaagtcggaatcgctagtaatcgtggatcagaatgccacggtgaatacgttcccgggccttgtacacaccgcccgtcacaccatgggagtgggttgcaaaagaagtaggtagcttaaccttcgggagggcgcttaccactttgtgattcatgactggggtgaagtcgtaacaaggtaaccgtaggggaacctgcggttggatcacgagactaccttaaagaagcgtactttgtagtgctcacacagattgtctgatagaaagtgaaaagcaaggcgtttacgcgttgggagtgaggctgaagagaataaggccgttcgctttctattaatgaaagctcaccctacacgaaaatatcacgcaacgcgtgataagcaattttcgtgtccccttcgtctagaggcccaggacaccgccctttcacggcggtaacaggggttcgaatcccctaggggacgccacttgctggtttgtgagtgaaagtcgccgaccttaatatctcaaaactcatcttcgggtgatgtttgagatatttgctctttaaaaatctggatcaagctgaaaattgaaacactgaacaacgagagttgttcgtgagtctctcaaattttcgcaacacgatgatgaatcgaaagaaacatcttcgggttgtgaggttaagcgactaagcgtacacggtggatgccctggcagtcagaggcgatgaaggacgtgctaatctgcgataagcgtcggtaaggtgatatgaaccgttataaccggcgatttccgaatggggaaacccagtgtgtttcgacacactatcattaactgaatccataggttaatgaggcgaaccgggggaactgaaacatctaagtaccccgaggaaaagaaatcaaccgagattcccccagtagcggcgagcgaacggggagcagcccagagcctgaatcagtgtgtgtgttagtggaagcgtctggaaaggcgcgcgatacagggtgacagccccgtacacaaaaatgcacatgctgtgagctcgatgagtagggcgggacacgtggtatcctgtctgaatatggggggaccatcctccaaggctaaatactcctgactgaccgatagtgaaccagtaccgtgagggaaaggcgaaaagaaccccggcgaggggagtgaaaaagaacctgaaaccgtgtacgtacaagcagtgggagcacgcttgggtaccggctgggccgaccagaatcatgcaagtgcgtaagatagtcgcgggccggcccggccgggtactcaggcgtgtgactgcgtaccttttgtataatgggtcagcgacttatattctgtagcaaggttaaccgaataggggagccgaagggaaaccgagtcttaactgggcgttaagttgcagggtatagacccgaaacccggtgatctagccatgggcaggttgaaggttgggtaacactaactggaggaccgaaccgactaatgttgaaaaattagcggatgacttgtggctgggggtgaaaggccaatcaaaccgggagatagctggttctccccgaaagctatttaggtagcgcctcgtgaattcatctccgggggtagagcactgtttcggcaagggggtcatcccgacttaccaacccgatgcaaactgcgaataccggagaatgttatcacgggagacacacggcgggtgctaacgtccgtcgtgaagagggaaacaacccagaccgccagctaaggtcccaaagtcatggttaagtgggaaacgatgtgggaaggcccagacagccaggatgttggcttagaagcagccatcatttaaagaaagcgtaatagctcactggtcgagtcggcctgcgcggaagatgtaacggggctaaaccatgcaccgaagctgcggcagcgacgcttatgcgttgttgggtaggggagcgttctgtaagcctgcgaaggtgtgctgtgaggcatgctggaggtatcagaagtgcgaatgctgacataagtaacgataaagcgggtgaaaagcccgctcgccggaagaccaagggttcctgtccaacgttaatcggggcagggtgagtcgacccctaaggcgaggccgaaaggcgtagtcgatgggaaacaggttaatattcctgtacttggtgttactgcgaaggggggacggagaaggctatgttggccgggcgacggttgtcccggtttaagcgtgtaggctggttttccaggcaaatccggaaaatcaaggctgaggcgtgatgacgaggcactacggtgctgaagcaacaaatgccctgcttccaggaaaagcctctaagcatcaggtaacatcaaatcgtaccccaaaccgacacaggtggtcaggtagagaataccaaggcgcttgagagaactcgggtgaaggaactaggcaaaatggtgccgtaacttcgggagaaggcacgctgatatgtaggtgaggtccctcgcggatggagctgaaatcagtcgaagataccagctggctgcaactgtttattaaaaacacagcactgtgcaaacacgaaagtggacgtatacggtgtgacgcctgcccggtgccggaaggttaattgatggggttagcgcaagcgaagctcttgatcgaagccccggtaaacggcggccgtaactataacggtcctaaggtagcgaaattccttgtcgggtaagttccgacctgcacgaatggcgtaatgatggccaggctgtctccacccgagactcagtgaaattgaactcgctgtgaagatgcagtgtacccgcggcaagacggtaagaccccgtgaacctttactatagcttgacactgaacattgagccttgatgtgtaggataggtgggaggctttgaagtgtggacgccagtctgcatggagccgaccttgaaataccaccctttaatgtttgatgttctaacgttgacccgtaatccgggttgcggacagtgtctggtgggtagtttgactggggcggtctcctcctaaagagtaacggaggagcacgaaggttggctaatcctggtcggacatcaggaggttagtgcaatggcataagccagcttgactgcgagcgtgacggcgcgagcaggtgcgaaagcaggtcatagtgatccggtggttctgaatggaagggccatcgctcaacggataaaaggtactccggggataacaggctgataccgcccaagagttcatatcgacggcggtgtttggcacctcgatgtcggctcatcacatcctggggctgaagtaggtcccaagggtatggctgttcgccatttaaagtggtacgcgagctgggtttagaacgtcgtgagacagttcggtccctatctgccgtgggcgctggagaactgaggggggctgctcctagtacgagaggaccggagtggacgcatcactggtgttcgggttgtcatgccaatggcactgcccggtagctaaatgcggaagagataagtgctgaaagcatctaagcacgaaacttgccccgagatgagttctccctgaccctttaagggtcctgaaggaacgttgaagacgacgacgttgataggccgggtgtgtaagcgcagcgatgcgttgagctaaccggtactaatgaaccgtgaggcttaaccttacaacgccgaagctgttttggcggatgagagaagattttcagcctgatacagattaaatcagaacgcagaagcggtctgataaaacagaatttgcctggcggcagtagcgcggtggtcccacctgaccccatgccgaactcagaagtgaaacgccgtagcgccgatggtagtgtggggtctccccatgcgagagtagggaactgccaggcatcaaataaagctgagttggctgctgccaccgctgagcaataactagcataaccccttggggcctctaaacgggtcttgaggggttttttgctgaaaggaggaactatatccggattggcgaatgggacgcgccctgtagcggcgcattaagcgcggcgggtgtggtggttacgcgcagcgtgaccgctacacttgccagcgccctagcgcccgctcctttcgctttcttcccttcctttctcgccacgttcgccggctttccccgtcaagctctaaatcgggggctccctttagggttccgatttagtgctttacggcacctcgaccccaaaaaacttgattagggtgatggttcacgtagtgggccatcgccctgatagacggtttttcgccctttgacgttggagtccacgttctttaatagtggactcttgttccaaactggaacaacactcaaccctatctcggtctattcttttgatttataagggattttgccgatttcggcctattggttaaaaaatgagctgatttaacaaaaatttaacgcgaattttaacaaaatattaacgtttacaatttcaggtggcacttttcggggaaatgtgcgcggaacccctatttgtttatttttctaaatacattcaaatatgtatccgctcatgaattaattcttagaaaaactcatcgagcatcaaatgaaactgcaatttattcatatcaggattatcaataccatatttttgaaaaagccgtttctgtaatgaaggagaaaactcaccgaggcagttccataggatggcaagatcctggtatcggtctgcgattccgactcgtccaacatcaatacaacctattaatttcccctcgtcaaaaataaggttatcaagtgagaaatcaccatgagtgacgactgaatccggtgagaatggcaaaagtttatgcatttctttccagacttgttcaacaggccagccattacgctcgtcatcaaaatcactcgcatcaaccaaaccgttattcattcgtgattgcgcctgagcgagacgaaatacgcgatcgctgttaaaaggacaattacaaacaggaatcgaatgcaaccggcgcaggaacactgccagcgcatcaacaatattttcacctgaatcaggatattcttctaatacctggaatgctgttttcccggggatcgcagtggtgagtaaccatgcatcatcaggagtacggataaaatgcttgatggtcggaagaggcataaattccgtcagccagtttagtctgaccatctcatctgtaacatcattggcaacgctacctttgccatgtttcagaaacaactctggcgcatcgggcttcccatacaatcgatagattgtcgcacctgattgcccgacattatcgcgagcccatttatacccatataaatcagcatccatgttggaatttaatcgcggcctagagcaagacgtttcccgttgaatatggctcataacaccccttgtattactgtttatgtaagcagacagttttattgttcatgaccaaaatcccttaacgtgagttttcgttccactgagcgtcagaccccgtagaaaagatcaaaggatcttcttgagatcctttttttctgcgcgtaatctgctgcttgcaaacaaaaaaaccaccgctaccagcggtggtttgtttgccggatcaagagctaccaactctttttccgaaggtaactggcttcagcagagcgcagataccaaatactgtccttctagtgtagccgtagttaggccaccacttcaagaactctgtagcaccgcctacatacctcgctctgctaatcctgttaccagtggctgctgccagtggcgataagtcgtgtcttaccgggttggactcaagacgatagttaccggataaggcgcagcggtcgggctgaacggggggttcgtgcacacagcccagcttggagcgaacgacctacaccgaactgagatacctacagcgtgagctatgagaaagcgccacgcttcccgaagggagaaaggcggacaggtatccggtaagcggcagggtcggaacaggagagcgcacgagggagcttccagggggaaacgcctggtatctttatagtcctgtcgggtttcgccacctctgacttgagcgtcgatttttgtgatgctcgtcaggggggcggagcctatggaaaaacgccagcaacgcggcctttttacggttcctggccttttgctggccttttgctcacatgttctttcctgcgttatcccctgattctgtggataaccgtattaccgcctttgagtgagctgataccgctcgccgcagccgaacgaccgagcgcagcgagtcagtgagcgaggaagcggaagagcgcctgatgcggtattttctccttacgcatctgtgcggtatttcacaccgcatatatggtgcactctcagtacaatctgctctgatgccgcatagttaagccagtatacactccgctatcgctacgtgactgggtcatggctgcgccccgacacccgccaacacccgctgacgcgccctgacgggcttgtctgctcccggcatccgcttacagacaagctgtgaccgtctccgggagctgcatgtgtcagaggttttcacc